European Patent Specification EP 3 366 126 B1, published May 15, 2024. Title: TRANSGENIC MICE EXPRESSING HUMAN LAMBDA AND KAPPA IMMUNOGLOBULIN LIGHT CHAIN VARIABLE DOMAINS. Applicant: Kymab Limited. The sequence listing filed with the application follows.

SEQUENCE LISTING (68 sequences)

SEQ ID NO: 1 - DNA, 4272 bp, Rattus norvegicus
agatctgcccatctcaggctagttaaattagttcatcccagtttggcccaacttaccccatctagagtagcgaaactaatctgagcctagctaagtccagtttagtttaatgtagcccagcttggcacaggctaatacatactgctacagtttggtctagcctaccctaattaagctgatccaggcctgggtagacctagctcatctcagcccagttaaggttatccagtacatctctttccagttcagctcaggttaccataccttatctcaattcagctcagctagtgtaattcatcttagttcatcccctacccctctagactccctgttgatcttaactcagtttagacatggccaacaaagcctggcccaactcaggccaggttagtgtagctcagcataagcagtctagccttgctcagtctagctcacccttcctcatctaaattcaactcagctatgccggccctgcagcaggtcccctcagctcacccaagtccaaccagttcagtctggctcatttaagtcttgacaatccccaattcatcccagctcagcttagcataactcaggcagtccattcttagcccaacccagtttagcccagtttatcccagttcatcctggctgtactcagtgcaactcgattcatgttctcccaggccacctcagcccagttcatggtagctcatctgagcccaacttatcccagctcatcccaaaccacctcacctaagccctgctcagcctagctcatctgagcctagttcaacctctctcatcctgccagctagcccagtttagtccacatcatcttgcaaagctcaaccagcccaagtcagccgggtccagctcattcatgtccaaaccagctcagtcatgctcatcctaactcagcctcaccatcatccacatcagctagcccagttcagctgagctcatcccagcccacttcaatcacagctcatttaagtacagctcaccccagctctatttagctcaagctagcttatttagcctacttcatcccagctcagcccagccaactcaactcatcctagctcagctaaaccctgctcagctcacccaagcaaagctgactccaacccagatcctttcagctcagctcacccagctcaggccagctcacccatcccagctcacccagcttagctcacccagcccagctcagcccagctcacccagcccagctcagcccagctcacccagcccagctcagcccagctcagctcagctcagctcagctcagctcagctcacccagctcagctcagccagctcagctcaccccagctcagtccagctcagttcagctcaccccagctcagctcacccaactcagctcactcaactcagctcacccaactcagctcagctcagttcacccagctcagctcacccagcccagcacagctcatctcacccagctcagctcacccagcccagctcaccccagctcaccccagctcagctcagctcaccccagctcagcccagctcagctcacccagctcagctcacccaactcagctcagctcagttcacccagctcagctcacccagcccagcacagctcatctcacccagcccagctcaccccagctcaccccagctcagctcagctcagcccagctcacccagctcagctcagctcaccccagctcagctcacccagctcagctcacccagcccagctcagctcagctcaccccagctcagcccagctcagctcacccagctcagctcacccagcccagctcaccccagctcaccccagctcagtccagctcagttcagctcacccagctcagctcacccaactcaactcagctcagttcacccagctcagctcagctcaccccagctcaccccagctcacccagctcagttcagctcaccccagctcagttcacccagctcagctcacccagcccagctcagcccagctcaccccagctcagctcaaccagatcagctcagcccagctcaccctagtttagttcacccagcccagctcaccccagctcagctcaccccaactcagctcacccagctcatcccagctcagccagctaatcccagctcagctcaccccagctcagctcacccagctcagctcacccaactcagctcaccccagctcaccccagctcatcccagctcatcccagttcagacctgttcagctcatctcaccccagctcagctcaccccagttcagctcacctagcccaactcaccccagctcagtccagctcagttcagctcaccccaactcatctcacccagctcagctcaccccagctcatcccagctcagctcaccccagttcagccctgttcagctcatctcacccagctcagctcatccagcccagctcaccccagctcaccccagctcagtccagctcagttcagctcacccagctcagctcacccaactcaactcagctcagttcacccagctcagctcagctcaccccagctcacccagctcagttcagctcaccccagctcagttcacccagctcagctcacccagcccagctcaaccagatcagctcagcccagctcaccctagtttagttcacccagcccagctcaccccagctcagctcaccccaactcagctcacctagctcatcccagctcagctcaccccagctcagctcaccccagctcatctcaccccagctcagctcacccagctcatcccagctcagctcagcccagctcatcccagccctgctcatcccagctcagctcagctcagcccagctcagcccagctcagcccagctcagcccagctcagcccagctcagctcaacccagctcagctcacccagcccagctcagcccagctcacccagctcagctcaccccagctcagctcaccccagctcatctcacccagctcagctcacccagctcagcccagctcagctcagctcacccagctcatctcacccagctcagctcaccccagctcatcccagctcagctcaccccagttcagccctgttcagctcatctcaccccagctcagctcacccagttcagctcatcccagcccatcccagctcagctcagcccagctcagcccagctcagcccagcccagcccagcccagctcagctcagcccagctcagcccagctcagtccagctcagcttagcccagcccagctcagctcagcccagctcagcccagctcagcccagctcagctcacccagctcaccccagctcagcccagctcagcccagctcagctcacccagctcaccccaccccagctcaccccagttcagcccagctcagcccagctcagcccagcccagcccagcccagcccagcccagctcagcccagctcagctcagcccagcccagctcagctcagcccagctcagcccagctcatcccagctcagctcaccccagctcagcccagctcagcccagctcagctcacccagctcaccccaccccagctcaccccagttcagcccagctcatccagctcagctcacccccagctctgctcacccagctcagctcagcttacccagctcagctcaactcacccagctcagctcacccagctcagctcagctcaccccagcccagctcagctcagctcaccccagctctgctcacccagctcagctcagctcacctcagctctgctcacccagctcagctcaaccacctcaggtcagcccagctcaccccagcttaccccagctcacccagctcagctcagctcacccagctcagctcacccagctcagctcaccccagcttaccccagctcaccccagctcagctaacccagctcagctcacccagctcagctcacccagctcagctcatcccagctcaccccagctaccacagagtagctcatgctagctcagctcaccccagcacaacacagcccaacacagctcagttcagagcagtccagtagagtttagctccaatcagcccagatcaagacaattcattccaatttggctatcttggttaagtcagcctagtttagcttagccggcctagctcaattcagctcattgcagtctacctcgttcctgctcaagtccagctttggctacctcagagtaatcatctcagcttagcacatttttgaagggctcagggaagcctacacatctcagtccaactgtgcttaactagagcctagcttcctagccaggctgtcaaccttgttcactaaattttgctcagcaagctt

SEQ ID NO: 2 - DNA, 22190 bp, Artificial Sequence
  Tragetting Vector (long version)
gcggccgcaacctgggcaaatgggagcttagcaacaatgtagggggctggacctagacttcctacacatttgtagcagatgtgcagcttggtcttcatgtgtgtattaccctaacatttggagcaggagctgtctctgactctgttgcctgccattggatccccttcccctgcttgggctgccttgtttggccttagtaggaaaggatgtgcttagtcctgctgtgacttgatgtccctaggcagaatgataccccaggggggctccccatctctgaggagatgggcaaagggtaatggttggagggacttgtgaggctgggactgggaggagagaaaggagacagctgtaactggaatgatgttaagtgaacaaatgaatggatagattagatagacagatagacagacagacagacagacagacagacagacagacagacagatagaaagatagatagataaggggaaaaagaaacgtagctgagcaagccagagagagcaagccaaataagcagcattcctccatgacttttccttcagctcctgcctatgagtctgccttgacttccctcagtgattggttgtaagttaaaaggtgaaataaaccctttctttgacaagttgcttttggttctgatttttatcacagcaagagaaaatcaaactagaacaaacatgtatttttcctggcacatgtccatagtaaggcagaaatgatcttcagacctagaccatagatactacagagagcagaagtgtagataggtggacttactgtatgattgtaatccaagtaaatctacatagctagagagctagaggaaaggccaaagcttcctctgggaggtcagatcctgtcgcactgtagccaataaggcatattgcatcacaggaaaggactaagacccaggctggcaatagtgtctgtatcttaactagacctctctagtgagtgaggaaggaagtttgtgagagcccagactgtgggctcggaaggtacctgccatgcccctgttagtaactgagtactacagcaggagcaggtgttctctagaaagcctgagacaactctacttcttctctcaagagaccacctaatacaggcctgagagaacagactctggaaatagatgggacttaaggagctaagatctagagctcatctacagagcagaatcccagccaagagaacaaagaatactggctctctctcctgttccctactcctagagttctaaaacacactatagggaagggagcctctagacctccgtccattccccatcttgctcattccatcttcccatgtccccaggtctccaagccacagacactacctttcctattcacccacctttctgtgtccctaggtccccaggccatagtcacctccccccacacacaccccactcaccctgccccatctatgcccctagatgcttacttaccagagtcttttgtctgacgtggggctacaagcatctatgctccctaagcacctactgctgacctgtaggacccagctctgaaccaactcatataagtaaatacagactctcccctgtcttaggatggcctcctggatcaggaggagaccactgccaaagaaccttctctcagagcactgaactcctcccctgtaccacttaggacagacctgagacctattattactgattaccagagctctggcagtgaccacggaggagataggtccaccctggacacaggaaacacagcagcagagatactgctccatcacaacagtagagtgacactttagactttaatttgggtcactttcctgctgcagaggtgggatcagaaagcaaagagcagtatgagtgcctgataggcacccaagtacactatagagtactcatggtgaataaggtacctccatggcttcccagggaggggcactgccccacccccaccatcacagacctttctccatagttgataactcagacacaagtgaatgacagatggacctccatctactcttattttaaaaagaagacaaaccccacaggctcgagaactttagcgactgttttgagagaaatcattggtccctgactcaagagatgactggcagattggggatcagaatacccatactctgtggctagtgtgaggtttaagcctcagagtccctgtggtctctgactggtgcaaggttttgactaagcggagcaccacagtgctaactgggaccacggtgacacgtggctcaacaaaaaccttctgtttggagctctccaggggcagcctgagctatgaggaagtagagaggcttgagaaatctgaggaagaaaagagtagatctgagaggaaaggtagctttctggaggtcaggagacagtgcagagaagaacgagttactgtggacaggtcttagatggggaaagaatgagcaaatgcaagcatcagaagggtggatgcaatgtcctgccaaggacttaccaagaggatccccggacagagcaggcaggtggagttgactgagaggacagggtaggtgcaggtccctctctcgtttcctttctccttctcctgtttccttcctctcttgtcacaggtctcactatgctagccaaggctagcctgaaagattaccatcctacagatgggcccatccagttgagttaaggtggagatctctccaaacatctgagtttctgaggcttggatgccactggggacgccaagggactttgggctgggtttggttggccccagatgaagggctacttcactgggtctataattactctgatgtctaggaccagggggctcaggtcactcaggtcaggtgagtcctgcatctggggactgtggggttcaggtgtcctaaggcaggatgtggagagagttttagtataggaacagaggcagaacagagactgtgctactggtacttcgatgtctggggcgcagggaccacggtcaccgtctcctcaggtaagctggcttttttctttctgcacattccattctgaaatgggaaaagatattctcagatctccccatgtcaggccatctgccacactctgcatgctgcagaagcttttctgtaaggatagggtcttcactcccaggaaaagaggcagtcagaggctagctgcctgtggaacagtgacaatcatggaaaataggcatttacattgttaggctacatgggtagatgggtttttgtacacccactaaaggggtctatgatagtgtgactactttgactactggggccaaggcaccactctcacagtctcctcaggtgagtccttacaacctctctcttctattcagcttaaatagattttactgcatttgttgggggggaaatgtgtgtatctgaatttcaggtcatgaaggactagggacaccttgggagtcagaaagggtcattgggagccctggctgatgcagacagacatcctcagctcccagacttcatggccagagatttatagggatcctggccagcattgccgctaggtccctctcttctatgctttctttgtccctcactggcctccatctgagatcatcctggagccctagccaaggatcatttattgtcaggggtctaatcattgttgtcacaatgtgcctggtttgcttactggggccaagggactctggtcactgtctctgcaggtgagtcctaacttctcccattctaaatgcatgttggggggattctgagccttcaggaccaagattctctgcaaacgggaatcaagattcaacccctttgtcccaaagttgagacatgggtctgggtcagggactctctgcctgctggtctgtggtgacattagaactgaagtatgatgaaggatctgccagaactgaagcttgaagtctgaggcagaatcttgtccagggtctatcggactcttgtgagaattaggggctgacagttgatggtgacaatttcagggtcagtgactgtctggtttctctgaggtgaggctggaatataggtcaccttgaagactaaagaggggtccaggggcttctgcacaggcagggaacagaatgtggaacaatgacttgaatggttgattcttgtgtgacaccaggaattggcataatgtctgagttgcccaggggtgattctagtcagactctggggtttttgtcgggtatagaggaaaaatccactattgtgattactatgctatggactactggggtcaaggaacctcagtcaccgtctcctcaggtaagaatggcctctccaggtctttatttttaacctttgttatggagttttctgagcattgcagactaatcttggatatttgtccctgagggagccggctgagagaagttgggaaataaactgtctagggatctcagagcctttaggacagattatctccacatctttgaaaaactaagaatctgtgtgatggtgttggtggagtccctggatgatgggatagggactttggaggctcatttgagggagatgctaaaacaatcctatggctggagggatagttggggctacgcgtttttaaccctagaaagatagtctgcgtaaaattgacgcatgcattcttgaaatattgctctctctttctaaatagcgcgaatccgtcgctgtgcatttaggacatctcagtcgccgcttggagctcccgtgaggcgtgcttgtcaatgcggtaagtgtcactgattttgaactataacgaccgcgtgagtcaaaatgacgcatgattatcttttacgtgacttttaagatttaactcatacgataattatattgttatttcatgttctacttacgtgataacttattatatatatattttcttgttatagatatcgctagtggatccggctggttctttccgcctcagaaggtacttttttttttttttttttttttttttttttttttttttttttttttttttttttttttttaaatttttgggaatttattgatttgcatttaaaagggaactgctgacaaagattcactggtaataatttgaacaagttggaaaatacagtcaacattactgaaacactactaaaataattccaggacagaacaaaacttcttagatgctgtctttgatgtgaaaattgactgcttcttacttttctaacacacggtggtataattaacaatattcaatcacttctattctttcctgcatatataaaaattaaaataccaattaaaaaactaatatatcttctctttatttcttacagatatgagttcaatgtttcactcaatagtgctgtggtttaagagaattttttcatttacaagttaaacaacaatccgcccaaagggaactgatagtctataggctcatagtgcaaataaacagtttaggaatgcagcaactgacatttctaaagtacaaaacagataaaattcttagaagatacatgcaaaaagctctactaagcagatggccacagaactagaacattgataattttactggcgatgtcaataggactccagatgtttccaaactcaacttgaactctcatcttaggctttgtattttgcttttccagtttcactaatgacacaaacatgattcaaatccctgaagtattcattatagtcaagggcatatcctacaacaaacttgtctggaatttcaaatccaacaaagtctggcttatatccaacacttcgtggggtccttttcaccagcaagcttgcgaccttgaccatctttggattatactgcctgaccaaggaaagcaaagtctgcattgttttgccagtgtcaattatatcttccacaatcaagacattctttccagttaaagttgagagatcatctccaccaattacttttatgtcccctgttgactggtcattacaatagctcttcagtctgataaaatctacagtcataggaatggatctatcactatttctattcagtgctttgatgtaatccagcaggtcagcaaagaatttatagccccccttgagcacacagagggctacaatgtgatggcctcccatctccttcatcacatctcgagcaagacgttcagtcctacagaaataaaatcaggaatttaatagaaagtttcatacattaaactttataacaaacacctcttagtcattaaacttccacaccaacctgggcaatatagtgagaccccatgcctgcaaaaaaaaaaaaattagccaggcatggtagcatgtacctgtagtcccagctacttgagaggtgaggtgggaaaatcactttagtgcaggatgttgaggctggagtgaactgtgattgtgccactgcactccagcctggacaatagagcaagaccttgtctcaaaaaaatgcattaaaaattttttttaaatcttccacgtaacacatcctttgccctcatgtttcataaggtaaaaaatttgataccttcaaaaaaaccaagcataccactatcataattttttttaaatgcaaataaaaacaagataccattttcacctatcagactggcaggttctgattaaatgaaatttcttggataatatacaatattaagagagactgtagaaactgggccagtggctcatgcctgtaatcccagcactttgggaggctgggtaacatggcgaaccctgtttctacaaaataaaaatattagctgggagtggtggcgcacacctatagtcccagctactcaggaggctgaggtggaaggatcgcttgaacccaggaggttgagactgcagtgaactgtgatcattctgctgcactgcaccccagcctgggcaacagagaccttgtctcaaaaaaaaaaaaaaaagagacaaattgtgaagagaaaggtactctcatataacatcaggagtataaaatgattcaacttcttagaggaaaatttggcaataccaaaatattcaataaactctttccccttgacccagaaattccacttgaataaagctgaacaagtaccaaacatgtaaaagaatgtttcttctagtacagtcggtaagaacaaaatagtgtctatcaatagtggactggttaaatcagttatggtatctccataagacagaatgctatgcaacctttaaaatatattagatagctctagacagtggatcccctcgagggacctaataacttcgtatagcatacattatacgaagttatattaagggttattgaatatgtcgactagacacactaatattaaaagtgtccaataacatttaaaactatactcatacgttaaaatataaatgtatatatgtacttttgcatatagtatacatgcatagccagtgcttgagaagaaatgtgtacagaaggctgaaaggagagaactttagtcttcttgtttatggcctccatagttagaatattttataacacaaatattttgatattataattttaaaataaaaacacagaatagccagacatacaatgcaagcattcaataccaggtaaggtttttcactgtaattgacttaacagaaaattttcaagctagatgtgcataataataaaaatctgaccttgccttcatgtgattcagccccagtccattaccctgtttaggactgagaaatgcaagactctggctagagttccttcttccatctcccttcaatgtttactttgttctggtccctacagagtcccactataccacaactgatactaagtaattagtaaggccctcctcttttatttttaataaagaagattttagaaagcatcagttatttaataagttggcctagtttatgttcaaatagcaagtactcagaacagctgctgatgtttgaaattaacacaagaaaaagtaaaaaacctcattttaagatcttacttacctgtccataattagtccatggggaataaacaccctttccaaatcctcagcataatgattaggtatgcaaaataaatcaaggtcataacctggttcatcatcactaatcacgacgccagggctgcgggtcgccataacggagccggccggcgcgcgggctgaataacttcgtataatgtgtactatacgaagttatttgttcaggaggaggaagccggtggcggagcagaggaggaggcggaggcgcagcaagacccccccccccctgcaggtcgaaaggcccggagatgaggaagaggagaacagcgcggcagacgtgcgcttttgaagcgtgcagaatgccgggcctccggaggaccttcgggcgcccgccccgcccctgagcccgcccctgagcccgcccccggacccaccccttcccagcctctgagcccagaaagcgaaggagcaaagctgctattggccgctgccccaaaggcctacccgcttccattgctcagcggtgctgtccatctgcacgagactagtgagacgtgctacttccatttgtcacgtcctgcacgacgcgagctgcggggcgggggggaacttcctgactaggggaggagtagaaggtggcgcgaaggggccaccaaagaacggagccggttggcgcctaccggtggatgtggaatgtgtgcgaggccagaggccacttgtgtagcgccaagtgcccagcggggctgctaaagcgcatgctccagactgccttgggaaaagcgcctcccctacccggtagatatctataacaagaaaatatatatataataagttatcacgtaagtagaacatgaaataacaatataattatcgtatgagttaaatcttaaaagtcacgtaaaagataatcatgcgtcattttgactcacgcggtcgttatagttcaaaatcagtgacacttaccgcattgacaagcacgcctcacgggagctccaagcggcgactgagatgtcctaaatgcacagcgacggattcgcgctatttagaaagagagagcaatatttcaagaatgcatgcgtcaattttacgcagactatctttctagggttaaaagaattcgatatcaagcttatcgatgtagttggagattttcagtttttagaataaaagtattagttgtggaatatacttcaggaccacctctgtgacagcatttatacagtatccgatgcatagggacaaagagtggagtggggcactttctttagatttgtgaggaatgttccgcactagattgtttaaaacttcatttgttggaaggagagctgtcttagtgattgagtcaagggagaaaggcatctagcctcggtctcaaaagggtagttgctgtctagagaggtctggtggagcctgcaaaagtccagctttcaaaggaacacagaagtatgtgtatggaatattagaagatgttgcttttactcttaagttggttcctaggaaaaatagttaaatactgtgactttaaaatgtgagagggttttcaagtactcatttttttaaatgtccaaaatttttgtcaatcaatttgaggtcttgtttgtgtagaactgacattacttaaagtttaaccgaggaatgggagtgaggctctctcataccctattcagaactgacttttaacaataataaattaagtttaaaatatttttaaatgaattgagcaatgttgagttggagtcaagatggccgatcagaaccagaacacctgcagcagctggcaggaagcaggtcatgtggcaaggctatttggggaagggaaaataaaaccactaggtaaacttgtagctgtggtttgaagaagtggttttgaaacactctgtccagccccaccaaaccgaaagtccaggctgagcaaaacaccacctgggtaatttgcatttctaaaataagttgaggattcagccgaaactggagaggtcctcttttaacttattgagttcaaccttttaattttagcttgagtagttctagtttccccaaacttaagtttatcgacttctaaaatgtatttagaattcattttcaaaattaggttatgtaagaaattgaaggactttagtgtctttaatttctaatatatttagaaaacttcttaaaattactctattattcttccctctgattattggtctccattcaattcttttccaatacccgaagcatttacagtgactttgttcatgatcttttttagttgtttgttttgccttactattaagactttgacattctggtcaaaacggcttcacaaatctttttcaagaccactttctgagtattcattttaggagaaatactttttttttaaatgaatgcaattatctagacttatttcagttgaacatgctggttggtggttgagaggacactcagtcagtcagtgacgtgaagggcttctaagccagtccacatgctctgtgtgaactccctctggccctgcttattgttgaatgggccaaaggtctgagaccaggctgctgctgggtaggcctggactttgggtctcccacccagacctgggaatgtatggttgtggcttctgccacccatccacctggctgctcatggaccagccagcctcggtggctttgaaggaacaattccacacaaagactctggacctctccgaaaccaggcaccgcaaatggtaagccagaggcagccacagctgtggctgctgctcttaaagcttgtaaactgtttctgcttaagagggactgagtcttcagtcattgctttagggggagaaagagacatttgtgtgtcttttgagtaccgttgtctgggtcactcacatttaactttccttgaaaaactagtaaaagaaaaatgttgcctgttaaccaataatcatagagctcatggtattttgaggaaatcttagaaaacgtgtatacaattgtctggaattatttcagttaagtgtattagttgaggtactgatgctgtctctacttcagttatacatgtgggtttgaattttgaatctattctggctcttcttaagcagaaaatttagataaaatggatacctcagtggtttttaatggtgggtttaatatagaaggaatttaaattggaagctaatttagaatcagtaaggagggacccaggctaagaaggcaatcctgggattctggaagaaaagatgtttttagtttttatagaaaacactactacattcttgatctacaactcaatgtggtttaatgaatttgaagttgccagtaaatgtacttcctggttgttaaagaatggtatcaaaggacagtgcttagatccaaggtgagtgtgagaggacaggggctggggtatggatacgcagaaggaaggccacagctgtacagaattgagaaagaatagagacctgcagttgaggccagcaggtcggctggactaactctccagccacagtaatgacccagacagagaaagccagactcataaagcttgctgagcaaaatttagtgaacaaggttgacagcctggctaggaagctaggctctagttaagcacagttggactgagatgtgtaggcttccctgagcccttcaaaaatgtgctaagctgagatgattactctgaggtagccaaagctggacttgagcaggaacgaggtagactgcaatgagctgaattgagctaggccggctaagctaaactaggctgacttaaccaagatagccaaattggaatgaattgtcttgatctgggctgattggagctaaactctactggactgctctgaactgagctgtgttgggctgtgttgtgctggggtgagctgagctagcatgagctactctgtggtagctggggtgagctgggatgagctgagctgggtgagctgagctgggtgagctgagctgggttagctgagctggggtgagctggggtaagctggggtgagctgagctgggtgagctgagctgggtgagctgagctgagctgggtgagctggggtaagctggggtgagctgggctgacctgaggtggttgagctgagctgggtgagcagagctgaggtgagctgagctgagctgggtgagcagagctggggtgagctgagctgagctgggctggggtgagctgagctgagctgggtgagctgagctgggtgagttgagctgagctgggtaagctgagctgagctgggtgagcagagctgggggtgagctgagctggatgagctgggctgaactggggtgagctggggtggggtgagctgggtgagctgagctgggctgagctgggctgagctggggtgagctgagctgggatgagctgggctgagctgggctgagctgagctgggctgggctgagctgagctgggctgagctgggctgggctgggctgggctgggctgggctgagctgggctgagctgggctgaactggggtgagctggggtggggtgagctgggtgagctgagctgggctgagctgggctgagctggggtgagctgggtgagctgagctgggctgagctgggctgagctgggctgagctgagctgggctgggctaagctgagctggactgagctgggctgagctgggctgagctgagctgggctgggctgggctgggctgagctgggctgagctgggctgagctgagctgggatgggctgggatgagctgaactgggtgagctgagctggggtgagatgagctgaacagggctgaactggggtgagctgagctgggatgagctggggtgagctgagctgggtgagatgagctgggtgagctgagctgagctgggctgagctgggtgagctgagctgggtgagatgagctggggtgagctgagctggggtgagctgagctgggtgagctgggctgagctgggctgggtgagctgagctgggttgagctgagctgggctgagctgggctgagctgggctgagctgggctgagctgggctgagctgagctgagctgggatgagcagggctgggatgagctgggctgagctgagctgggatgagctgggtgagctgagctggggtgagatgagctggggtgagctgagctggggtgagctgagctgggatgagctaggtgagctgagttggggtgagctgagctggggtgagctgggctgggtgaactaaactagggtgagctgggctgagctgatctggttgagctgggctgggtgagctgagctgggtgaactgagctggggtgagctgaactgagctgggtgagctggggtgagctgagctgagctgggtgaactgagctgagttgagttgggtgagctgagctgggtgagctgaactgagctggactgagctggggtgagctggggtgagctgggctggatgagctgagctgggtgagatgagctgaacagggctgaactggggtgagctgagctgggatgagctggggtgagctgagctgggtgagatgagttggggtgagctgaactgagctggactgagctggggtgagttgggctaggtgagctgaactggggtgagctgagctggggtgagatgagctgaacaggtctgaactgggatgagctgggatgagctggggtgagctggggtgagctgagttgggtgagctgagctgggtgagctgagctggggtgagctgagctgggattagctggctgagctgggatgagctgggtgagctgagttggggtgagctgagctggggtgagctgggctgggtgaactaaactagggtgagctgggctgagctgatctggttgagctgagctggggtgagctgggctgagctgggctgggtgagctgagctgggtgaactgagctggggtgagctgaactgagctgggtgagctggggtgagctggggtgagctgagctgagctgggtgaactgagctgagttgagttgggtgagctgagctgggtgagctgaactgagctggactgagctggggtgagctggggtgagctgggctgggtgagctgagctgggtgagctgagctgggctgagctggggtgagctgagctgagctgggctgggtgagctgagctgggtgagctgagctggggtgagctgagctgagctgggtgagctgggctgagctgagctgagctggggtgagctggggtgagctgggctgggtgagatgagctgtgctgggctgggtgagctgagctgggtgaactgagctgagctgagttgggtgagctgagctgggtgagctgagctgggctgagctggggtgagctgagctgagctggggtgagctggggtgagctgggctgggtgagctgagctgggtgagatgagctgtgctgggctgggtgagctgagctgggtgaactgagctgagctgagttgggtgagctgagttgagtgagctgagttgggtgagctgagctggggtgagctgaactgagctggactgagctggggtgagctgagctggctgagctgagctgggtgagctgagctgagctgagctgagctgagctgagctgggctgagctgggctgggtgagctgggctgagctgggctgggtgagctgggctgagctgggctgggtgagctaagctgggtgagctgggatgggtgagctggcctgagctgggtgagctgagctgaaaggatctgggttggagtcagctttgcttgggtgagctgagcagggtttagctgagctaggatgagttgagttggctgggctgagctgggatgaagtaggctaaataagctagcttgagctaaatagagctggggtgagctgtacttaaatgagctgtgattgaagtgggctgggatgagctcagctgaactgggctagctgatgtggatgatggtgaggctgagttaggatgagcatgactgagctggtttggacatgaatgagctggacccggctgacttgggctggttgagctttgcaagatgatgtggactaaactgggctagctggcaggatgagagaggttgaactaggctcagatgagctaggctgagcagggcttaggtgaggtggtttgggatgagctgggataagttgggctcagatgagctaccatgaactgggctgaggtggcctgggagaacatgaatcgagttgcactgagtacagccaggatgaactgggataaactgggctaaactgggttgggctaagaatggactgcctgagttatgctaagctgagctgggatgaattggggattgtcaagacttaaatgagccagactgaactggttggacttgggtgagctgaggggacctgctgcagggccggcatagctgagttgaatttagatgaggaagggtgagctagactgagcaaggctagactgcttatgctgagctacactaacctggcctgagttgggccaggctttgttggccatgtctaaactgagttaagatcaacagggagtctagaggggtaggggatgaactaagatgaattacactagctgagctgaattgagataaggtatggtaacctgagctgaactggaaagagatgtactggataaccttaactgggctgagatgagctaggtctacccaggcctggatcagcttaattagggtaggctagaccaaactgtagcagtatgtattagcctgtgccaagctgggctacattaaactaaactggacttagctaggctcagattagtttcgctactctagatggggtaagttgggccaaactgggatgaactaatttaactagcctgagatgggcagatctgaatgagcagagctgggatgaactgaatgagtttcaccaggcctggaccagttaggctaggacctcgttctatagaggcagactgtgtgctacagtggagtttcaagatgattccatgagtcctccccgcccccaacataacccaccttcctcctaccctacaagcctgtctggtgtgtaaatcccagctttgtgtgctgatacagaagcctgagcccctcccccacctccacctacctattactttgggatgagaatagttctcccagccagtgtctcagagggaagccaagcaggacaggcccaaggctacttgagaagccaggatctaggcctctccctgagaacgggtgttcatgcccctagagttggctgaagggccagatccacctactctagaggcatctctccctgtctgtgaaggcttccaaagtcacgttcctgtggctagaaggcagctccatagccctgctgcagtttcgtcctgtataccaggttcacctactaccatatctagccctgcctgccttaagagtagcaacaaggaaatagcagggtgtagagggatctcctgtctgacaggaggcaagaagacagattcttacccctccatttctcttttatccctctctggtcctcagagagtcagtccttcccaaatgtcttccccctcgtctcctgcgagagccccctgtctgataagaatctggtggccatgggctgcctggcccgggacttcctgcccagcaccatttccttcacctggaactaccagaacaacactgaagtcatccagggtatcagaaccttcccaacactgaggacagggggcaagtacctagccacctcgcaggtgttgctgtctcccaagagcatccttgaaggttcagatgaatacctggtatgcaaaatccactacggaggcaaaaacaaagatctgcatgtgcccattccaggtaagaaccaaaccctcccagcaggggtgcccaggcccaggcatggcccagagggagcagcggggtggggcttaggccaagctgagctcacaccttgacctttcattccagctgtcgcagagatgaaccccaatgtaaatgtgttcgtcccaccacgggatggcttctctggccctgcaccacgcaagtctaaactcatctgcgaggccacgaacttcactccaaaaccgatcacagtatcctggctaaaggatgggaagctcgtggaatctggcttcaccacagatccggtgaccatcgagaacaaaggatccacaccccaaacctacaaggtcataagcacacttaccatctctgaaatcgactggctgaacctgaatgtgtacacctgccgtgtggatcacaggggtctcaccttcttgaagaacgtgtcctccacatgtgctgccagtgagtggcctgggataagcccaatgcctagccctcccagattagggaagtcctcctacaattatggccaatgccacccagacatggtcatttgctccttgaactttggctccccagagtggccaaggacaagaatgagcaataggcagtagaggggtgagaatcagctggaaggaccagcatcttcccttaagtaggtttgggggatggagactaagcttttttccaacttcacaactagatatgtcataacctgacacagtgttctcttgactgcaggtccctccacagacatcctaaccttcaccatccccccctcctttgccgacatcttcctcagcaagtccgctaacctgacctgtctggtctcaaacctggcaacctatgaaaccctgaatatctcctgggcttctcaaagtggtgaaccactggaaaccaaaattaaaatcatggaaagccatcccaatggcaccttcagtgctaagggtgtggctagtgtttgtgtggaagactggaataacaggaaggaatttgtgtgtactgtgactcacagggatctgccttcaccacagaagaaattcatctcaaaacccaatggtaggtatccccccttcccttcccctccaattgcaggacccttcctgtacctcatagggagggcaggtcctcttccaccctatcctcactactgtcttcatttacagaggtgcacaaacatccacctgctgtgtacctgctgccaccagctcgtgagcaactgaacctgagggagtcagccacagtcacctgcctggtgaagggcttctctcctgcagacatcagtgtgcagtggcttcagagagggcaactcttgccccaagagaagtatgtgaccagtgccccgatgccagagcctggggccccaggcttctactttacccacagcatcctgactgtgacagaggaggaatggaactccggagagacctatacctgtgttgtaggccacgaggccctgccacacctggtgaccgagaggaccgtggacaagtccactggtaaacccacactgtacaatgtctccctgatcatgtctgacacaggcggcacctgctattgaccatgctagcgctcaaccaggcaggccctgggtgtccagttgctctgtgtatgcaaactaaccatgtcagagtgagatgttgcattttataaaaattagaaataaaaaaaatccattcaaacgtcactggttttgattatacaatgctcatgcctgctgagacagttgtgttttgcttgctctgcacacaccctgcatacttgcctccaccctggcccttcctctaccttgccagtttcctccttgtgtgtgaactcagtcaggcttacaacagacagagtatgaacatgcgattcctccagctacttctagatatatggctgaaagcttgcctaacctggtgcaggcagcattcaggcacatatatagacacacatgcatttatacatagatatataggtacacatgtgtagacacatacatgaatgtgtattcatggacacacagacaaaggtacacatatatacacatgagttcatgcgcacacacatgcatggacacttacaaacgccttcagagacaaataggcatagacacacaaccactcacagaaacagataccaatatgcatggtcctgtgtacacagaaacagactataggcaaatatacacaaataaactatatagatacaaagatatgcatatacacacatgtacagaaacatcttcacatgtgtacactaacatgtggacaggtatagcacacagatacacctggactctgaccagggctgtaatctccaaggctcacggctcagagagcctacactaggctgggtcactgatactcctcaggagcccactctatgattgggagagataaccccaggtacaaagtatgcctatctgtctcaacaccatggggcagaagatactccactaaccacccatgacagaaagttagccttggctgtgtctccattaatagaacacctcagaagaccaatgtgaaattgcctaacccactcacacccaccctgatctccagttcaaaatgcagaaaacataatgcagttgtccaaaagatgccccaaccacacacacacacacacacacacacacacacacacacacacacacacacatacacacacacacaccatcaaggagcctctgtaaggagtcaccacccaataacactgcctctttgggctcatatcctggacattcttcatattcatatccatttggggcctaggctttagatatccccaagggctcatctttacagggatcagagatcccaataaatgccctggtcccacagcctccctcaggtatctgtctgtttatctcttggtacctttcttagacgttaggtggcacttttcggggaaatgtgcgcggaacccctatttgtttatttttctaaatacattcaaatatgtatccgctcatgagacaataaccctgataaatgcttcaataatattgaaaaaggaagagtatgagtattcaacatttccgtgtcgcccttattcccttttttgcggcattttgccttcctgtttttgctcacccagaaacgctggtgaaagtaaaagatgctgaagatcagttgggtgcacgagtgggttacatcgaactggatctcaacagcggtaagatccttgagagttttcgccccgaagaacgttttccaatgatgagcacttttaaagttctgctatgtggcgcggtattatcccgtgttgacgccgggcaagagcaactcggtcgccgcatacactattctcagaatgacttggttgagtactcaccagtcacagaaaagcatcttacggatggcatgacagtaagagaattatgcagtgctgccataaccatgagtgataacactgcggccaacttacttctgacaacgatcggaggaccgaaggagctaaccgcttttttgcacaacatgggggatcatgtaactcgccttgatcgttgggaaccggagctgaatgaagccataccaaacgacgagcgtgacaccacgatgcctgcagcaatggcaacaacgttgcgcaaactattaactggcgaactacttactctagcttcccggcaacaattaatagactggatggaggcggataaagttgcaggaccacttctgcgctcggcccttccggctggctggtttattgctgataaatctggagccggtgagcgtgggtctcgcggtatcattgcagcactggggccagatggtaagccctcccgtatcgtagttatctacacgacggggagtcaggcaactatggatgaacgaaatagacagatcgctgagataggtgcctcactgattaagcattggtaactgtcagaccaagtttactcatatatactttagattgatttaaaacttcatttttaatttaaaaggatctaggtgaagatcctttttgataatctcatgaccaaaatcccttaacgtgagttttcgttccactgagcgtcagaccccgtagaaaagatcaaaggatcttcttgagatcctttttttctgcgcgtaatctgctgcttgcaaacaaaaaaaccaccgctaccagcggtggtttgtttgccggatcaagagctaccaactctttttccgaaggtaactggcttcagcagagcgcagataccaaatactgtccttctagtgtagccgtagttaggccaccacttcaagaactctgtagcaccgcctacatacctcgctctgctaatcctgttaccagtggctgctgccagtggcgataagtcgtgtcttaccgggttggactcaagacgatagttaccggataaggcgcagcggtcgggctgaacggggggttcgtgcacacagcccagcttggagcgaacgacctacaccgaactgagatacctacagcgtgagctatgagaaagcgccacgcttcccgaagggagaaaggcggacaggtatccggtaagcggcagggtcggaacaggagagcgcacgagggagcttccagggggaaacgcctggtatctttatagtcctgtcgggtttcgccacctctgacttgagcgtcgatttttgtgatgctcgtcaggggggcggagcctatggaaaaacgccagcaacgcggcctttttacggttcctggccttttgctggccttttgctcacatgttctttcctgcgttatcccctgattctgtggataaccgtattaccgcctttgagtgagctgataccgctcgccgcagccgaacgaccgagcgcagcgagtcagtgagcgaggaagcggaagagcgcctgatgcggtattttctccttacgcatctgtgcggtatttcacaccgcatatggtgcactctcagtacaatctgctctgatgccgcatagttaagccagtatacactccgctatcgctacgtgactgggtcatggctgcgccccgacacccgccaacacccgctgacgcgccctgacgggcttgtctgctcccggcatccgcttacagacaagctgtgaccgtctccgggagctgcatgtgtcagaggttttcaccgtcatcaccgaaacgcgcgaggcagctgcggtaaagctcatcagcgtggtcgtgaagcgattcacagatgtctgcctgttcatccgcgtccagctcgttgagtttctccagaagcgttaatgtctggcttctgataaagcgggccatgttaagggcggttttttcctgtttggtcactgatgcctccgtgtaagggggatttctgttcatgggggtaatgataccgatgaaacgagagaggatgctcacgatacgggttactgatgatgaacatgcccggttactggaacgttgtgagggtaaacaactggcggtatggatgcggcgggaccagagaaaaatcactcagggtcaatgccagcgcttcgttaatacagatgtaggtgttccacagggtagccagcagcatcctgcgatgcagatccggaacataatggtgcagggcgctgacttccgcgtttccagactttacgaaacacggaaaccgaagaccattcatgttgttgctcaggtcgcagacgttttgcagcagcagtcgcttcacgttcgctcgcgtatcg

SEQ ID NO: 3 - DNA, 14130 bp, Artificial Sequence
  Targetting vector (short version)
gcggccgcaacctgggcaaatgggagcttagcaacaatgtagggggctggacctagacttcctacacatgtgtaacagatgtgcagcttggtcttcatgtgtgtattaccctaacatttggagcaggagctgtctctgactctgttgcctgccattggatccccttcccctgcttgggctgccttgtttggccttagtaggaaaggatgtgcttagtcctgctgtgacttgatgtccctaggcagaatgataccccaggggggctccccatctctgaggagatgggcaaagggtaatggttggagggacttgtgaggctgggactgggaggagagaaaggagacagctgtaactggaatgatgttaagtgaacaaatgaatggatagattagatagacagatagacagacagacagacagacagacagacagacagacagacagacagatagaaagatagatagataaggggaaaaagaaacgtagctgagcaagccagagagagcaagccaaataagcagcattcctccatgacttttccttcagctcctgcctatgagtctgccttgacttccctcagtgattggttgtaagttaaaaggtgaaataaaccctttctttgacaagttgcttttggttctgatttttatcacagcaagagaaaatcaaactagaacaaacatgtatttttcctggcacatgtccatagtaaggcagaaatgatcttcagacctagaccatagatactacagagagcagaagtgtagataggtggacttactgtatgattgtaatccaagtaaatctacatagctagagagctagaggaaaggccaaagcttcctctgggaggtcagatcctgtcgcactgtagccaataaggcatattgcatcacaggaaaggactaagacccaggctggcaatagtgtctgtatcttaactagatctctctagtgagtgaggaagtaaatttgtgagagcccagactgtgggctcggaaggtacctgccatgcccctgttagtaactgagtactacagcaggagcaggtgttctctagaaagcctgagacaactctacttcttctctcaagagaccacctaatacaggcctgagagaacagactctggaaatagatgggacttacggagctaagatctagagctcatctacagagcagaatcccagccaagagaacaaagaatactgactctctcctgttccctactcctagagttctaaaacacactatagggaagggagcctctagacctccgtccattccccatcttgctcattccatcttcccatgtccccaggtctccaagccacagacaccacctttcctattcacccacctttctgtgtccctaggtccccaggccatagtcacctccccccacaccccgctcaccctgccccatctatgcccctagatgcttacttaccagagtcttttgtctgacgtggggctacaagcatctatgctccctaagcacctactgctgacctgtaggacccagctctgaaccaactcatataagtaaatacagactctcccctgtcttaggatggccccctgggtcaggaggagaccactgccaaggaaccttctcttagagcactgaactcctcccctgtaccacttaggacagacctgagacctattattactgattaccagagctctggcagtgaccacggaggagatagatccaccctggacacaggaaacacagcaccagagatactgcttcatcacaacagtagagtgacactttagactttaatttgggtcactttcctgctgtagaggtgggatcagaaagcaaagagcagtatgagtgcctgataggcacccaagtacactatagagtactcatggtgaataaggtacctccatggcttcccagggaggggcactgccccacccccaccatcacagacctttctccatagttgataactcagacacaagtgaatgacagatggacctccatctgctcttattttaaaaagaagacaaaccccacaggctcgagaactttagcgactgttttgagagaaatcattggtccctgactcaagagatgactggcagattggggatcagaatacccatactctgtggctagtgtgaggtttaagcctcagagtccctgtggtctctgactggtgcaaggttttgactaagcggagcaccacagtgctaactgggaccacggtgacacgtggctcaacaaaaaccttctgtttggagctctccaggggcagcctgagctatgaggaagtagagaggcttgagaaatctgaggaagaaaagagtagatctgagaggaaaggtagctttctggaggtcaggagacagtgcagagaagaacgagttactgtggacaggtcttagatggggaaagaatgagcaaatgcaagcatcagaagggtggatgcaatgtcctgccaaggacttaccaagaggatccccggacagagcaggcaggtggagttgactgagaggacaggataggtgcaggtccctctcttgtttcctttctccttctcctgtttccttcttctcttgtcacaggtctcactatgctagccaaggctagcctgaaagattaccatcctacagatgggcccatccagttgaattaaggtggagatctctccaaacatctgagtttctgaggcttggatgccactggggacgccaagggactttgggatgggtttggttggccccagatgaagggctacttcactgggtctataattactctgatgtctaggaccagggggctcaggtcactcaggtcaggtgagtcctgcatctggggactgtggggttcaggtggcctaaggcaggatgtggagagagttttagtataggaacagaggcagaacagagactgtgctactggtacttcgatgtctggggcacagggaccacggtcaccgtctcctcaggtaagctggcttttttctttctgcacattccattctgaaacgggaaaagatattctcagatctccccatgtcaggccatctgccacactctgcatgctgcagaagcttttctgtaaggatagggtcttcactcccaggaaaagaggcagtcagaggctagctgcctgtggaacagtgacaatcatggaaaataggcatttacattgttaggctacatgggtagatgggtttttgtacacccactaaaggggtctatgatagtgtgactactttgactactggggccaaggcaccactctcacagtctcctcaggtgagtccttacaacctctctcttctattcagcttaaatagattttactgcatttgttgggggggaaatgtgtgtatctgaatttcaggtcatgaaggactagggacaccttgggagtcagaaagggtcattgggagccctggctgacgcagacagacatcctcagctcccatacttcatggccagagatttatagggatcctggccagcattgccgctaggtccctctcttctatgctttctttgtccctcactggcctccatctgagatcatcctggagccctagccaaggatcatttattgtcaggggtctaatcattgttgtcacaatgtgcctggtttgcttactggggccaagggactctggtcactgtctctgcaggtgagtcctaacttctcccattctaaatgcatgttggggggattctgggccttcaggaccaagattctctgcaaacgggaatcaagattcaacccctttgtcccaaagttgagacatgggtctgggtcagggactctctgcctgctggtctgtggtgacattagaactgaagtatgatgaaggatctgccagaactgaagcttgaagtctgaggcagaatcttgtccagggtctatcggactcttgtgagaattaggggctgacagttgatggtgacaatttcagggtcagtgactgtctggtttctctgaggtgaggctggaatataggtcaccttgaagactaaagaggggtccaggggcttctgcacaggcagggaacagaatgtggaacaatgacttgaatggttgattcttgtgtgacaccaggaattggcataatgtctgagttgcccaggggtgattctagtcagactctggggtttttgtcgggtatagaggaaaaatccactattgtgattactatgctatggactactggggtcaaggaacctcagtcaccgtctcctcaggtaagaatggcctctccaggtctttatttttaacctttgttatggagttttctgagcattgcagactaatcttggatatttgtccctgagggagccggctgagagaagttgggaaataaactgtctagggatctcagagcctttaggacagattatctccacatctttgaaaaactaagaatctgtgtgatggtgttggtggagtccctggatgatgggatagggactttggaggctcatttgaagaagatgctaaaacaatcctatggctggagggatagttggggctacgcgtttttaaccctagaaagatagtctgcgtaaaattgacgcatgcattcttgaaatattgctctctctttctaaatagcgcgaatccgtcgctgtgcatttaggacatctcagtcgccgcttggagctcccgtgaggcgtgcttgtcaatgcggtaagtgtcactgattttgaactataacgaccgcgtgagtcaaaatgacgcatgattatcttttacgtgacttttaagatttaactcatacgataattatattgttatttcatgttctacttacgtgataacttattatatatatattttcttgttatagatatcgctagtggatcctggttctttccgcctcagaaggtacttttttttttttttttttttttttttttttttttttttttttttttttttttttttttttaaatttttgggaatttattgatttgcatttaaaagggaactgctgacaaagattcactggtaataatttgaacaagttggaaaatacagtcaacattactgaaacactactaaaataattccaggacagaacaaaacttcttagatgctgtctttgatgtgaaaattgactgcttcttacttttctaacacacggtggtataattaacaatattcaatcacttctattctttcctgcatatataaaaattaaaataccaattaaaaaactaatatatcttctctttatttcttacagatatgagttcaatgtttcactcaatagtgctgtggtttaagagaattttttcatttacaagttaaacaacaatccgcccaaagggaactgatagtctataggctcatagtgcaaataaacagtttaggaatgcagcaactgacatttctaaagtacaaaacagataaaattcttagaagatacatgcaaaaagctctactaagcagatggccacagaactagaacattgataattttactggcgatgtcaataggactccagatgtttccaaactcaacttgaactctcatcttaggctttgtattttgcttttccagtttcactaatgacacaaacatgattcaaatccctgaagtattcattatagtcaagggcatatcctacaacaaacttgtctggaatttcaaatccaacaaagtctggcttatatccaacacttcgtggggtccttttcaccagcaagcttgcgaccttgaccatctttggattatactgcctgaccaaggaaagcaaagtctgcattgttttgccagtgtcaattatatcttccacaatcaagacattctttccagttaaagttgagagatcatctccaccaattacttttatgtcccctgttgactggtcattacaatagctcttcagtctgataaaatctacagtcataggaatggatctatcactatttctattcagtgctttgatgtaatccagcaggtcagcaaagaatttatagccccccttgagcacacagagggctacaatgtgatggcctcccatctccttcatcacatctcgagcaagacgttcagtcctacagaaataaaatcaggaatttaatagaaagtttcatacattaaactttataacaaacacctcttagtcattaaacttccacaccaacctgggcaatatagtgagaccccatgcctgcaaaaaaaaaaaaattagccaggcatggtagcatgtacctgtagtcccagctacttgagaggtgaggtgggaaaatcactttagtgcaggatgttgaggctggagtgaactgtgattgtgccactgcactccagcctggacaatagagcaagaccttgtctcaaaaaaatgcattaaaaattttttttaaatcttccacgtaacacatcctttgccctcatgtttcataaggtaaaaaatttgataccttcaaaaaaaccaagcataccactatcataattttttttaaatgcaaataaaaacaagataccattttcacctatcagactggcaggttctgattaaatgaaatttcttggataatatacaatattaagagagactgtagaaactgggccagtggctcatgcctgtaatcccagcactttgggaggctgggtaacatggcgaaccctgtttctacaaaataaaaatattagctgggagtggtggcgcacacctatagtcccagctactcaggaggctgaggtggaaggatcgcttgaacccaggaggttgagactgcagtgaactgtgatcattctgctgcactgcaccccagcctgggcaacagagaccttgtctcaaaaaaaaaaaaaaaagagacaaattgtgaagagaaaggtactctcatataacatcaggagtataaaatgattcaacttcttagaggaaaatttggcaataccaaaatattcaataaactctttccccttgacccagaaattccacttgaataaagctgaacaagtaccaaacatgtaaaagaatgtttcttctagtacagtcggtaagaacaaaatagtgtctatcaatagtggactggttaaatcagttatggtatctccataagacagaatgctatgcaacctttaaaatatattagatagctctagacagtggatcccctcgagggacctaataacttcgtatagcatacattatacgaagttatattaagggttattgaatatgtcgactagacacactaatattaaaagtgtccaataacatttaaaactatactcatacgttaaaatataaatgtatatatgtacttttgcatatagtatacatgcatagccagtgcttgagaagaaatgtgtacagaaggctgaaaggagagaactttagtcttcttgtttatggcctccatagttagaatattttataacacaaatattttgatattataattttaaaataaaaacacagaatagccagacatacaatgcaagcattcaataccaggtaaggtttttcactgtaattgacttaacagaaaattttcaagctagatgtgcataataataaaaatctgaccttgccttcatgtgattcagccccagtccattaccctgtttaggactgagaaatgcaagactctggctagagttccttcttccatctcccttcaatgtttactttgttctggtccctacagagtcccactataccacaactgatactaagtaattagtaaggccctcctcttttatttttaataaagaagattttagaaagcatcagttatttaataagttggcctagtttatgttcaaatagcaagtactcagaacagctgctgatgtttgaaattaacacaagaaaaagtaaaaaacctcattttaagatcttacttacctgtccataattagtccatggggaataaacaccctttccaaatcctcagcataatgattaggtatgcaaaataaatcaaggtcataacctggttcatcatcactaatcacgacgccagggctgcgggtcgccataacggagccggccggcgcgcgggctgaataacttcgtataatgtgtactatacgaagttatttgttcaggaggaggaagccggtggcggagcagaggaggaggcggaggcgcagcaagacccccccccccctgcaggtcgaaaggcccggagatgaggaagaggagaacagcgcggcagacgtgcgcttttgaagcgtgcagaatgccgggcctccggaggaccttcgggcgcccgccccgcccctgagcccgcccctgagcccgcccccggacccaccccttcccagcctctgagcccagaaagcgaaggagccaaagctgctattggccgctgccccaaaggcctacccgcttccattgctcagcggtgctgtccatctgcacgagactagtgagacgtgctacttccatttgtcacgtcctgcacgacgcgagctgcggggcgggggggaacttcctgactaggggaggagtagaaggtggcgcgaaggggccaccaaagaacggagccggttggcgcctaccggtggatgtggaatgtgtgcgaggccagaggccacttgtgtagcgccaagtgcccagcggggctgctaaagcgcatgctccagactgccttgggaaaagcgcctcccctacccggtagatatctataacaagaaaatatatatataataagttatcacgtaagtagaacatgaaataacaatataattatcgtatgagttaaatcttaaaagtcacgtaaaagataatcatgcgtcattttgactcacgcggtcgttatagttcaaaatcagtgacacttaccgcattgacaagcacgcctcacgggagctccaagcggcgactgagatgtcctaaatgcacagcgacggattcgcgctatttagaaagagagagcaatatttcaagaatgcatgcgtcaattttacgcagactatctttctagggttaaaagaattcgtagttggagattttcagtttttagaataaaagtattagctgcggaatatacttcaggaccacctctgtgacagcatttatacagtatccgatgcatagggacaaagagtggagtggggcactttctttagatttgtgaggaatgttccacactagattgtttaaaacttcatttgttggaaggagagctgtcttagtgattgagtcaagggagaaaggcatctagcctcggtctcaaaagggtagttgctgtctagagaggtctggtggagcctgcaaaagtccagctttcaaaggaacacagaagtatgtgtatggaatattagaagatgttgcttttactcttaagttggttcctaggaaaaatagttaaatactgtgactttaaaatgtgagagggttttcaagtactcatttttttaaatgtccaaaatttttgtcaatcaatttgaggtcttgtttgtgtagaactgacattacttaaagtttaaccgaggaatgggagtgaggctctctcataccctattcagaactgacttttaacaataataaattaagtttaaaatatttttaaatgaattgagcaatgttgagttggagtcaagatggccgatcagaaccagaacacctgcagcagctggcaggaagcaggtcatgtggcaaggctatttggggaagggaaaataaaaccactaggtaaacttgtagctgtggtttgaagaagtggttttgaaacactctgtccagccccaccaaaccgaaagtccaggctgagcaaaacaccacctgggtaatttgcatttctaaaataagttgaggattcagccgaaactggagaggtcctcttttaacttattgagttcaaccttttaattttagcttgagtagttctagtttccccaaacttaagtttatcgacttctaaaatgtatttagaattcattttcaaaattaggttatgtaagaaattgaaggactttagtgtctttaatttctaatatatttagaaaacttcttaaaattactctattattcttccctctgattattggtctccattcaattcttttccaatacccgaagcatttacagtgactttgttcatgatcttttttagttgtttgttttgccttactattaagactttgacattctggtcaaaacggcttcacaaatctttttcaagaccactttctgagtattcattttaggagaaatactttttttttaaatgaatgcaattatctagacttatttcggttgaacatgctggttggtggttgagaggacactcagtcagtcagtggcgtgaagggcttctaagccagtccacatgctctgtgtgaactccctctggccctgcttattgttgaatgggccaaaggtctgagaccaggctgctgctgggtaggcctggactttgggtctcccacccagacctgggaatgtatggttgtggcttctgccacccatccacctggctgctcatggaccagccagcctcggtggctttgaaggaacaattccacacaaagactctggacctctccgaaaccaggcaccgcaaatggtaagccagaggcagccacagctgtggctgctgctcttaaagcttgtaaactgtttctgcttaagagggactgagtcttcagtcattgctttagggggagaaagagacatttgtgtgtcttttgagtaccgttgtctgggtcactcacatttaactttccttgaaaaactagtaaaagaaaaatgttgcctgttaaccaataatcatagagctcatggtattttgaggaaatcttagaaaacgtgtatacaattgtctggaattatttcagttaagtgtattagttgaggtactgatgctgtctctacttcagttatacatgtgggtttgaattttgaatctattctggctcttcttaagcagaaaatttagataaaatggatacctcagtggtttttaatggtgggtttaatatagaaggaatttaaattggaagctaatttagaatcagtaaggagggacccaggctaagaaggcaatcctgggattctggaagaaaagatgtttttagtttttatagaaaacactactacattcttgatctacaactcaatgtggtttaatgaatttgaagttgccagtaaatgtacttcctggttgttaaagaatggtatcaaaggacagtgcttagatccaaggtgagtgtgagaggacaggggctggggtatggatacgcagaaggaaggccacagctgtacagaattgagaaagaatagagacctgcagttgaggccagcaggtcggctggactaactctccagccacagtaatgacccagacagagaaggccagactcataaagctttatcgataccgtcgacctcgagggggggcccggtacctttcttagacgtcaggtggcacttttcggggaaatgtgcgcggaacccctatttgtttatttttctaaatacattcaaatatgtatccgctcatgagacaataaccctgataaatgcttcaataatattgaaaaaggaagagtatgagtattcaacatttccgtgtcgcccttattcccttttttgcggcattttgccttcctgtttttgctcacccagaaacgctggtgaaagtaaaagatgctgaagatcagttgggtgcacgagtgggttacatcgaactggatctcaacagcggtaagatccttgagagttttcgccccgaagaacgttttccaatgatgagcacttttaaagttctgctatgtggcgcggtattatcccgtgttgacgccgggcaagagcaactcggtcgccgcatacactattctcagaatgacttggttgagtactcaccagtcacagaaaagcatcttacggatggcatgacagtaagagaattatgcagtgctgccataaccatgagtgataacactgcggccaacttacttctgacaacgatcggaggaccgaaggagctaaccgcttttttgcacaacatgggggatcatgtaactcgccttgatcgttgggaaccggagctgaatgaagccataccaaacgacgagcgtgacaccacgatgcctgcagcaatggcaacaacgttgcgcaaactattaactggcgaactacttactctagcttcccggcaacaattaatagactggatggaggcggataaagttgcaggaccacttctgcgctcggcccttccggctggctggtttattgctgataaatctggagccggtgagcgtgggtctcgcggtatcattgcagcactggggccagatggtaagccctcccgtatcgtagttatctacacgacggggagtcaggcaactatggatgaacgaaatagacagatcgctgagataggtgcctcactgattaagcattggtaactgtcagaccaagtttactcatatatactttagattgatttaaaacttcatttttaatttaaaaggatctaggtgaagatcctttttgataatctcatgaccaaaatcccttaacgtgagttttcgttccactgagcgtcagaccccgtagaaaagatcaaaggatcttcttgagatcctttttttctgcgcgtaatctgctgcttgcaaacaaaaaaaccaccgctaccagcggtggtttgtttgccggatcaagagctaccaactctttttccgaaggtaactggcttcagcagagcgcagataccaaatactgtccttctagtgtagccgtagttaggccaccacttcaagaactctgtagcaccgcctacatacctcgctctgctaatcctgttaccagtggctgctgccagtggcgataagtcgtgtcttaccgggttggactcaagacgatagttaccggataaggcgcagcggtcgggctgaacggggggttcgtgcacacagcccagcttggagcgaacgacctacaccgaactgagatacctacagcgtgagctatgagaaagcgccacgcttcccgaagggagaaaggcggacaggtatccggtaagcggcagggtcggaacaggagagcgcacgagggagcttccagggggaaacgcctggtatctttatagtcctgtcgggtttcgccacctctgacttgagcgtcgatttttgtgatgctcgtcaggggggcggagcctatggaaaaacgccagcaacgcggcctttttacggttcctggccttttgctggccttttgctcacatgttctttcctgcgttatcccctgattctgtggataaccgtattaccgcctttgagtgagctgataccgctcgccgcagccgaacgaccgagcgcagcgagtcagtgagcgaggaagcggaagagcgcctgatgcggtattttctccttacgcatctgtgcggtatttcacaccgcatatggtgcactctcagtacaatctgctctgatgccgcatagttaagccagtatacactccgctatcgctacgtgactgggtcatggctgcgccccgacacccgccaacacccgctgacgcgccctgacgggcttgtctgctcccggcatccgcttacagacaagctgtgaccgtctccgggagctgcatgtgtcagaggttttcaccgtcatcaccgaaacgcgcgaggcagctgcggtaaagctcatcagcgtggtcgtgaagcgattcacagatgtctgcctgttcatccgcgtccagctcgttgagtttctccagaagcgttaatgtctggcttctgataaagcgggccatgttaagggcggttttttcctgtttggtcactgatgcctccgtgtaagggggatttctgttcatgggggtaatgataccgatgaaacgagagaggatgctcacgatacgggttactgatgatgaacatgcccggttactggaacgttgtgagggtaaacaactggcggtatggatgcggcgggaccagagaaaaatcactcagggtcaatgccagcgcttcgttaatacagatgtaggtgttccacagggtagccagcagcatcctgcgatgcagatccggaacataatggtgcagggcgctgacttccgcgtttccagactttacgaaacacggaaaccgaagaccattcatgttgttgctcaggtcgcagacgttttgcagcagcagtcgcttcacgttcgctcgcgtatcg

SEQ ID NO: 4 - DNA, 3551 bp, Mus musculus
  misc_feature (1399)..(1498): n is a, c, g, or t
aagcttgctgagcaaaattaagggaacaaggttgagagccctagtaagcgaggctctaaaaagcatggctgagctgagatgggtgggcttctctgagcgcttctaaaatgcgctaaactgaggtgattactctgaggtaagcaaagctgggcttgagccaaaatgaagtagactgtaatgaactggaatgagctgggccgctaagctaaactaggctggcttaaccgagatgagccaaactggaatgaacttcattaatctaggttgaatagagctaaactctactgcctacactggactgttctgagctgagatgagctggggtgagctcagctatgctacgctgtgttggggtgagctgatctgaaatgagctactctggagtagctgagatggggtgagatggggtgagctgagctgggctgagctggactgagctgagctagggtgagctgagctgggtgagctgagctaagctggggtgagctgagctgagcttgactgagctagggtgagctggactgagctggggtgagctgagctgagctggggtaagctgggatgagctggggtgagctgagctgagctggagtgagctgagctgggctgagctggggtgagctgggctgggctgagctggggtgagctgggctgagctggggtgagctgagctggggtgagctgagctgagctggggtgagctgagctgagctggggtgagctgagctggggtgagctgagctgagctgggctgagctgaggtgagctgagctggggtgagctgagctggggtgagctgagctgagctggggtaagctgggatgagctggggtgagctgagctgagctggagtgagctgagctgggctgagctgggctgagctggggtgagctgagctggggtgagctgagctgagctgggctgagctgaggtgagctgagctggggtgagctgagctgagctggggtgagctgagctgagctggggtgagctgagctggggtgagctgagctggggtgagctgagctgagctggggtgagctgagctggggtgagctgagctgagctggggtgagctgagctgagctggggtgagctgagctgagctgagctggggtgagctgagctgagctggggtgagctgagctgagctggggtgagctgagctggggtgagctgggctgagctgagctgggctgagctgagctgagctgagctgagctggggtgagctgagctgggctgagctggggtgagctgggctgagctggggtgagctgagctggggtgagctgagctgagctggggtgagctgagctgagctggggtgagctgagctggggtgagctgagctgagctgggctgagctgagctgagctggggtgagctgagctgagctnnnnnnnnnnnnnnnnnnnnnnnnnnnnnnnnnnnnnnnnnnnnnnnnnnnnnnnnnnnnnnnnnnnnnnnnnnnnnnnnnnnnnnnnnnnnnnnnnnnnagctgagctgagctgagctgagctgagctggggtgagctggggtgagctgagctggggtgagctgagctgagctggggtgagctgagctgagctgagctgagctgagctgagctgggtgagctgagctgagctgagctggggtgagctgagctggggtgagctgagctgagctggggtgagctgagctggggtgagctgagctgagctggggtgagctggggtgagctggggtgagctggggtgagctgagctgaactggggtgagctgggctgagctggggtgagctgagctgagctgggctgagctggggtgagctggggtgagctggggtgagctgagctgagctagggtgagctgagctgagctagggtgagctgagctgagctggggtgagctgagctgagctggggtgagctgagctgagctggggtgagctgagctgagctggggtgagctgagctgagctggggtgagcttggctgagctggggtgagctggggtgagctgagctggggtgagctggggtaagctgagctgagctggggtgagctgagctgagctggggtgagctggggtgagctgagctgagctgagctgggtgatctgagctgagctgagctgggtgagctgagctgagctgagctgggtgagctgagctgagctgagctgagctgggtgagctgagctgagctgagctgagctgagctgagctggggtgagctgggctgagctgagctgagctggggtgagctgagctgagctgagctgagctggggtgagctgggctgagctggggtgagctgggctgagctgagctgggtgagctgagctgaactgagctgagctgggtgagctgagctgagctgagctgggtgagctgagctgggctgagctgagctgggtgagctgagctgaactgagctgagctgggtgagctgagctgagctgagctgggtgagctgagctggggtgagctgagctgagctggggtgagctgagctgagctgagctgggtgagctgagctggggtgagctgagctgagctggggtgagctgagctgagctggggtgagctgagctgagctggggtgagctgagctgagctggggtgagctgagctagggtgaactgggctgggtgagctggagtgagctgagctgaggtgaactggggtgagccgggatgttttgagttgagctggggtaagatgagctgaactggggtaagatgggatgagctgtggtgaggggagctggattgaactgagctgtgtgagctgagctggggtcagctgagcaagagtgagtagagctggctggccagaaccagaatcaattaggctaagtgagccagattgcgctgggatcagctgtactcagatgagctgggatgaggtaggctgggatgagctgggctagctgacatggattatgtgaggctgagctagcatgggctggcctagctgatgagctaagcttgaatgaacggggctgagctggactcagatgtgctagactgagctgtactggatgatctggtgtagggtgatctggactcaactgggctggctgatgggatgccccaggttgaactaggctcagataagttaggctgagtagggcctggttgagatggttcgggatgagctgggaaaagatggactgggaccatgaactgggctgagctgggttgggagaccatgaattgagctgaactgagtgcagctgggataaactgggttgagctaagaatagactacctgaattgtgccaaactgggctgggatcaattggaaattatcaggatttagatgagccggactaaactatgctgagctggactggttggatgtgttgaactggcctgctgctgggctggcatagctgagttgaacttaaatgaggaaggatgagcaaggctagcctgcttgcatagagctgaactttagcctagcctgagctggaccagcctgagctgagtaggtctaaactgagttaaaaatcaacagggataatttaacagctaatttaacaagcctgaggtctgagatt

SEQ ID NO: 5 - DNA, 2484 bp, Mus musculus
aagcttgctgagcaaaattaagggaacaaggttgagagccctagtaagcgaggctctaaaaagcacagctgagctgagatgggtgggcttctctgagtgcttctaaaatgcgctaaactgaggtgattactctgaggtaagcaaagctgggcttgagccaaaatgaagtagactgtaatgaactggaatgagctgggccgctaagctaaactaggctggcttaaccgagatgagccaaactggaatgaacttcattaatctaggttgaatagagctaaactctactgcctacactggactgttctgagctgagatgagctggggtgagctcagctatgctacgctgtgttggggtgagctgatctgaaatgagatactctggagtagctgagatggggtgagatggggtgagctgagctgggctgagctagactgagctgagctagggtgagctgagctgggtgagctgagctaagctggggtgagctgagctgagcttggctgagctagggtgagctgggctgagctggggtgagctgagctgagctggggtaagctgggatgagctggggtgagctgagctgagctggagtgagctgagctgggctgagctggggtgagctgggctgagctgggctgagctgggctgagctggggtgagctgagctggggtgagctgagctgagctggggtgagctgagctgagctggggtgagctggggtgagctgagctggggtgagctgagctgagctggggtgagctgagctggggtgagctgagctgagctggggtgagctgagctgagctgagctgagctgagctggggtgagctgagctgagctgagctggggtgagctggggtgagctgagctgagctggagtgagctgagctgggctgagctggggtgagctgggctgagctggggtgagctgagctgagctgagctgagctggggtgagctgagctgagctggggtgagctgagctggggtgagctgggctgagctgagctgagctgagctgagctgagctgagctgagctgagctgagctgagctgagctgagctgagctgagctgagctgagctggggtgagctgagctgagctgggctgagctggggtgagctgggctgagctgggctgagctgggctgagctggggtgagctgagctggggtgagctgagctgagctgggctgagctgagctgagctggggtgagctgagctgagctggggtgagctgagctgagctgagctggggtgagctgagctgggctgagcagggctgagctggggtgagctgagctgagctggggtgagctgggctgagctgggctgagctgagctgagctgggctgagctgggctgagctgggctgagctgggctgagctgggctgagctggggtgagctgagctgagctggggtgagctggggtgagctgagctggggtgagctgagctggggtgagctgagctgagctggggtgagctgagctggggtgagctgagctgagctggggtgagctgagctgagctggggtgagctgagctagggtgaactgggctgggtgagctggagtgagctgagctgaggtgaactggggtgagccgggatgttttgagttgagctggggtaagatgagctgaactggggtaaactgggatgagctgtggtgagcggagctggattgaactgagctgtgtgagctgagctggggtcagctgagcaagagtgagtagagctggctggccagaaccagaatcaattaggctaagtgagccagattgtgctgggatcagctgtactcagatgagctgggatgaggtaggctgggatgagctgggctagctgacatggattatgtgaggctgagctagcatgggctggcctagctgatgagctaagcttgaatgagcggggctgagctggactcagatgtgctagactgagctgtactggatgatctggtgtagggtgatctggactcaactgggctggctgatgggatgcgccaggttgaactaggctcagataagttaggctgagtagggcctggttgagatggttcgggatgagctgggaaaagatggactcggaccatgaactgggctgagctgggttgggagaccatgaattgagctgaactgagtgcagctgggataaactgggttgagctaagaatagactacctgaattgtgccaaactcggctgggatcaattggaaattatcaggatttagatgagccggactaaactatgctgagctggactggttggatgtgttgaactggcctgctgctgggctggcatagctgagttgaacttaaatgaggaaggctgagcaaggctagcctgcttgcatagagctgaactttagcctagcctgagctggaccagcctgagctgagtaggtctaaactgagttaaaaatcaacagggataatttaacagctaatttaacaagcctgaggtctgagatt

SEQ ID NO: 6 - DNA, 4515 bp, Artificial Sequence
  5' homology arm of targetting vector
aacctgggcaaatgggagcttagcaacaatgtagggggctggacctagacttcctacacatgtgtaacagatgtgcagcttggtcttcatgtgtgtattaccctaacatttggagcaggagctgtctctgactctgttgcctgccattggatccccttcccctgcttgggctgccttgtttggccttagtaggaaaggatgtgcttagtcctgctgtgacttgatgtccctaggcagaatgataccccaggggggctccccatctctgaggagatgggcaaagggtaatggttggagggacttgtgaggctgggactgggaggagagaaaggagacagctgtaactggaatgatgttaagtgaacaaatgaatggatagattagatagacagatagacagacagacagacagacagacagacagacagacagacagacagatagaaagatagatagataaggggaaaaagaaacgtagctgagcaagccagagagagcaagccaaataagcagcattcctccatgacttttccttcagctcctgcctatgagtctgccttgacttccctcagtgattggttgtaagttaaaaggtgaaataaaccctttctttgacaagttgcttttggttctgatttttatcacagcaagagaaaatcaaactagaacaaacatgtatttttcctggcacatgtccatagtaaggcagaaatgatcttcagacctagaccatagatactacagagagcagaagtgtagataggtggacttactgtatgattgtaatccaagtaaatctacatagctagagagctagaggaaaggccaaagcttcctctgggaggtcagatcctgtcgcactgtagccaataaggcatattgcatcacaggaaaggactaagacccaggctggcaatagtgtctgtatcttaactagatctctctagtgagtgaggaagtaaatttgtgagagcccagactgtgggctcggaaggtacctgccatgcccctgttagtaactgagtactacagcaggagcaggtgttctctagaaagcctgagacaactctacttcttctctcaagagaccacctaatacaggcctgagagaacagactctggaaatagatgggacttacggagctaagatctagagctcatctacagagcagaatcccagccaagagaacaaagaatactgactctctcctgttccctactcctagagttctaaaacacactatagggaagggagcctctagacctccgtccattccccatcttgctcattccatcttcccatgtccccaggtctccaagccacagacaccacctttcctattcacccacctttctgtgtccctaggtccccaggccatagtcacctccccccacaccccgctcaccctgccccatctatgcccctagatgcttacttaccagagtcttttgtctgacgtggggctacaagcatctatgctccctaagcacctactgctgacctgtaggacccagctctgaaccaactcatataagtaaatacagactctcccctgtcttaggatggccccctgggtcaggaggagaccactgccaaggaaccttctcttagagcactgaactcctcccctgtaccacttaggacagacctgagacctattattactgattaccagagctctggcagtgaccacggaggagatagatccaccctggacacaggaaacacagcaccagagatactgcttcatcacaacagtagagtgacactttagactttaatttgggtcactttcctgctgtagaggtgggatcagaaagcaaagagcagtatgagtgcctgataggcacccaagtacactatagagtactcatggtgaataaggtacctccatggcttcccagggaggggcactgccccacccccaccatcacagacctttctccatagttgataactcagacacaagtgaatgacagatggacctccatctgctcttattttaaaaagaagacaaaccccacaggctcgagaactttagcgactgttttgagagaaatcattggtccctgactcaagagatgactggcagattggggatcagaatacccatactctgtggctagtgtgaggtttaagcctcagagtccctgtggtctctgactggtgcaaggttttgactaagcggagcaccacagtgctaactgggaccacggtgacacgtggctcaacaaaaaccttctgtttggagctctccaggggcagcctgagctatgaggaagtagagaggcttgagaaatctgaggaagaaaagagtagatctgagaggaaaggtagctttctggaggtcaggagacagtgcagagaagaacgagttactgtggacaggtcttagatggggaaagaatgagcaaatgcaagcatcagaagggtggatgcaatgtcctgccaaggacttaccaagaggatccccggacagagcaggcaggtggagttgactgagaggacaggataggtgcaggtccctctcttgtttcctttctccttctcctgtttccttcttctcttgtcacaggtctcactatgctagccaaggctagcctgaaagattaccatcctacagatgggcccatccagttgaattaaggtggagatctctccaaacatctgagtttctgaggcttggatgccactggggacgccaagggactttgggatgggtttggttggccccagatgaagggctacttcactgggtctataattactctgatgtctaggaccagggggctcaggtcactcaggtcaggtgagtcctgcatctggggactgtggggttcaggtggcctaaggcaggatgtggagagagttttagtataggaacagaggcagaacagagactgtgctactggtacttcgatgtctggggcacagggaccacggtcaccgtctcctcaggtaagctggcttttttctttctgcacattccattctgaaacgggaaaagatattctcagatctccccatgtcaggccatctgccacactctgcatgctgcagaagcttttctgtaaggatagggtcttcactcccaggaaaagaggcagtcagaggctagctgcctgtggaacagtgacaatcatggaaaataggcatttacattgttaggctacatgggtagatgggtttttgtacacccactaaaggggtctatgatagtgtgactactttgactactggggccaaggcaccactctcacagtctcctcaggtgagtccttacaacctctctcttctattcagcttaaatagattttactgcatttgttgggggggaaatgtgtgtatctgaatttcaggtcatgaaggactagggacaccttgggagtcagaaagggtcattgggagccctggctgacgcagacagacatcctcagctcccatacttcatggccagagatttatagggatcctggccagcattgccgctaggtccctctcttctatgctttctttgtccctcactggcctccatctgagatcatcctggagccctagccaaggatcatttattgtcaggggtctaatcattgttgtcacaatgtgcctggtttgcttactggggccaagggactctggtcactgtctctgcaggtgagtcctaacttctcccattctaaatgcatgttggggggattctgggccttcaggaccaagattctctgcaaacgggaatcaagattcaacccctttgtcccaaagttgagacatgggtctgggtcagggactctctgcctgctggtctgtggtgacattagaactgaagtatgatgaaggatctgccagaactgaagcttgaagtctgaggcagaatcttgtccagggtctatcggactcttgtgagaattaggggctgacagttgatggtgacaatttcagggtcagtgactgtctggtttctctgaggtgaggctggaatataggtcaccttgaagactaaagaggggtccaggggcttctgcacaggcagggaacagaatgtggaacaatgacttgaatggttgattcttgtgtgacaccaggaattggcataatgtctgagttgcccaggggtgattctagtcagactctggggtttttgtcgggtatagaggaaaaatccactattgtgattactatgctatggactactggggtcaaggaacctcagtcaccgtctcctcaggtaagaatggcctctccaggtctttatttttaacctttgttatggagttttctgagcattgcagactaatcttggatatttgtccctgagggagccggctgagagaagttgggaaataaactgtctagggatctcagagcctttaggacagattatctccacatctttgaaaaactaagaatctgtgtgatggtgttggtggagtccctggatgatgggatagggactttggaggctcatttgaagaagatgctaaaacaatcctatggctggagggatagttggggct

SEQ ID NO: 7 - DNA, 25 bp, Artificial Sequence
  Oligonucleotide HV2-5
agatcaccttgaaggagtctggtcc

SEQ ID NO: 8 - DNA, 25 bp, Artificial Sequence
  Oligonucleotide HV4-4
tggtgaagccttcggagaccctgtc

SEQ ID NO: 9 - DNA, 25 bp, Artificial Sequence
  Oligonucleotide HV1-3
cactagctatgctatgcattgggtg

SEQ ID NO: 10 - DNA, 25 bp, Artificial Sequence
  Oligonucleotide HV1-2
atggatcaaccctaacagtggtggc

SEQ ID NO: 11 - DNA, 25 bp, Artificial Sequence
  Oligonucleotide HV6-1
ggaaggacatactacaggtccaagt

SEQ ID NO: 12 - DNA, 25 bp, Artificial Sequence
  Oligonucleotide C
taggtacttgccccctgtcctcagt

SEQ ID NO: 13 - DNA, 25 bp, Artificial Sequence
  Oligonucleotide KV1-9
agcccagtgtgttccgtacagcctg

SEQ ID NO: 14 - DNA, 25 bp, Artificial Sequence
  Oligonucleotide KV1-8
atcctcattctctgcatctacagga

SEQ ID NO: 15 - DNA, 25 bp, Artificial Sequence
  Oligonucleotide KV1-6
ggtaaggatggagaacactggcagt

SEQ ID NO: 16 - DNA, 25 bp, Artificial Sequence
  Oligonucleotide KV1-5
ttagtagctggttggcctggtatca

SEQ ID NO: 17 - DNA, 25 bp, Artificial Sequence
  Oligonucleotide Ck
ctttgctgtcctgatcagtccaact

SEQ ID NO: 18 - DNA, 10 bp, Artificial Sequence
  Rat Switch
  repeat_region (1)..(10): Repeated 148 times
gagctgagct

SEQ ID NO: 19 - DNA, 10 bp, Artificial Sequence
  Rat Switch
  repeat_region (1)..(10): Repeat 25 times
ggggtggggt

SEQ ID NO: 20 - DNA, 10 bp, Artificial Sequence
  Rat Switch
  repeat_region (1)..(5): Repeat 82 times
gggctgggct

SEQ ID NO: 21 - protein, 6 aa, Artificial Sequence
  Antibody Sequence
  MISC_FEATURE (1)..(2): Xaa Xaa = PR, RT, or PW
XXTFGQ

SEQ ID NO: 22 - protein, 17 aa, Artificial Sequence
  Antibody Sequence
  MISC_FEATURE (1)..(2): Xaa Xaa= PR, RT, or PW
XXTFGQGTKVEIKRADA

SEQ ID NO: 23 - protein, 6 aa, Artificial Sequence
  Antibody Sequence
  MISC_FEATURE (1)..(2): Xaa Xaa = PR or PW
XXTFGQ

SEQ ID NO: 24 - protein, 17 aa, Artificial Sequence
  Antibody Sequence
  MISC_FEATURE (1)..(2): Xaa Xaa = PR or PW
XXTFGQGTKVEIKRADA

SEQ ID NO: 25 - DNA, 24 bp, Artificial Sequence
  Primer E1554
atgacttcagtgttgttctggtag

SEQ ID NO: 26 - DNA, 19 bp, Artificial Sequence
  Primer E1555
caccagattcttatcagac

SEQ ID NO: 27 - DNA, 35 bp, Artificial Sequence
  ELP1352_Cy1
agagcggccgctgggcaacgttgcaggtgacggtc

SEQ ID NO: 28 - DNA, 34 bp, Artificial Sequence
  ELP1353_Cy2b
agagcggccgctttgtccaccgtggtgctgctgg

SEQ ID NO: 29 - DNA, 33 bp, Artificial Sequence
  ELP1354_Cy2a
agagcggccgcacattgcaggtgatggactggc

SEQ ID NO: 30 - DNA, 35 bp, Artificial Sequence
  ELP1356_VH4-4
aggacgcgtgaaacacctgtggttcttcctcctgc

SEQ ID NO: 31 - DNA, 33 bp, Artificial Sequence
  ELP1357_VH1-2,3
aggacgcgtcaccatggactggacctggaggat

SEQ ID NO: 32 - DNA, 34 bp, Artificial Sequence
  ELP1358_VH6-1
aggacgcgtatgtctgtctccttcctcatcttcc

SEQ ID NO: 33 - DNA, 21 bp, Artificial Sequence
  mIgG1_2 rev
ggggccagtggatagacagat

SEQ ID NO: 34 - DNA, 18 bp, Artificial Sequence
  mIgG2b rev
cagtggatagactgatgg

SEQ ID NO: 35 - DNA, 18 bp, Artificial Sequence
  mIgG2a_2 rev
cagtggatagaccgatgg

SEQ ID NO: 36 - DNA, 20 bp, Artificial Sequence
  mCH1 unirev
  misc_feature (1)..(1): K = G or T
kcaggggccagtggatagac

SEQ ID NO: 37 - DNA, 20 bp, Artificial Sequence
  mCH1 unirev_2
  misc_feature (3)..(3): R = A or G
  misc_feature (6)..(6): Y = C or T
  misc_feature (12)..(12): M = A or C
tarccyttgacmaggcatcc

SEQ ID NO: 38 - protein, 24 aa, Artificial Sequence
  16C9
QEVINYYYYGMDVWGQGTTVTVSS

SEQ ID NO: 39 - protein, 24 aa, Artificial Sequence
  20B5
QEVINYYYYGMDVWGQGTTVTVSS

SEQ ID NO: 40 - protein, 26 aa, Artificial Sequence
  19F4
LEMATINYYYYGMDVWGQGTMVTVSS

SEQ ID NO: 41 - protein, 24 aa, Artificial Sequence
  19E1
QEFGNYYYYGMDVWGQGTTVTVSS

SEQ ID NO: 42 - protein, 24 aa, Artificial Sequence
  19G8
QEDGNPYYFGMDFWGQGTTVTVSS

SEQ ID NO: 43 - protein, 22 aa, Artificial Sequence
  20H10
GSSYYYDGMDVWGQGTTVTVSS

SEQ ID NO: 44 - protein, 25 aa, Artificial Sequence
  18D10
LENDYGYYYYGMDVWGQGTTVTVSS

SEQ ID NO: 45 - protein, 23 aa, Artificial Sequence
  16F2
RGGLSPLYGMDVWGQGTTVTVSS

SEQ ID NO: 46 - DNA, 15 bp, Artificial Sequence
  Rat Switch
gggctgggctgggct

SEQ ID NO: 47 - DNA, 20 bp, Artificial Sequence
  Rat Switch
gggctgggctgggctgggct

SEQ ID NO: 48 - DNA, 25 bp, Artificial Sequence
  Rat Switch
gggctgggctgggctgggctgggct

SEQ ID NO: 49 - DNA, 30 bp, Artificial Sequence
  Rat Switch
gggctgggctgggctgggctgggctgggct

SEQ ID NO: 50 - DNA, 10 bp, Artificial Sequence
  Rat Switch
  repeat_region (1)..(5): Repeat 6 to 81 times
gggctgggct

SEQ ID NO: 51 - protein, 6 aa, Artificial Sequence
  IGHV4-4*02  CDR1
SSNWWS

SEQ ID NO: 52 - protein, 6 aa, Artificial Sequence
  12D10 CDR1
SGNWWS

SEQ ID NO: 53 - protein, 6 aa, Artificial Sequence
  1283 CDR1
RSNWWS

SEQ ID NO: 54 - protein, 7 aa, Artificial Sequence
  IGHV6-1*01 CDR1
SNSAAWN

SEQ ID NO: 55 - protein, 7 aa, Artificial Sequence
  4A12 CDR1
SNSAAWN

SEQ ID NO: 56 - protein, 16 aa, Artificial Sequence
  IGHV4-4*02 CDR2
EIYHSGSTNYNPSLKS

SEQ ID NO: 57 - protein, 16 aa, Artificial Sequence
  12D10 CDR2
EIYHSGNTNYNPSLKS

SEQ ID NO: 58 - protein, 16 aa, Artificial Sequence
  1283 CDR2
EIYHSGSTNYNPSLKS

SEQ ID NO: 59 - protein, 18 aa, Artificial Sequence
  IGHV6-1*01 CDR2
RTYYRSKWYNDYAVSVKS

SEQ ID NO: 60 - protein, 18 aa, Artificial Sequence
  4A12 CDR2
RTYYRSKWYNDYKVSVKS

SEQ ID NO: 61 - protein, 12 aa, Artificial Sequence
  12D10 CDR3
GPLTGEKYYFDL

SEQ ID NO: 62 - protein, 8 aa, Artificial Sequence
  1283 CDR3
IGDWYFDL

SEQ ID NO: 63 - protein, 16 aa, Artificial Sequence
  4A12 CDR3
EGSHSGSGWYLDAFDI

SEQ ID NO: 64 - protein, 17 aa, Artificial Sequence
  IGHJ2*01 J-region
YWYFDLWGRGTLVTVSS

SEQ ID NO: 65 - protein, 16 aa, Artificial Sequence
  12D10 J-region
YYFDLWGRGTLVTVSS

SEQ ID NO: 66 - protein, 16 aa, Artificial Sequence
  1283 J-Region
WYFDLWGRGTLVTVSS

SEQ ID NO: 67 - protein, 16 aa, Artificial Sequence
  IGHJ3*01 J-Region
DAFDVWGQGTMVTVSS

SEQ ID NO: 68 - protein, 16 aa, Artificial Sequence
  4A12 J-region
DAFDIWGQGTKVTVSS